European Patent Application EP 4 410 820 A1, published August 7, 2024. Title: PEPTIDE HAVING ANTI-AGING ACTIVITY, AND USE THEREOF. Applicant: CAREGEN CO., LTD. Application KR. The sequence listing filed with the application follows.

SEQUENCE LISTING (9 sequences)

SEQ ID NO: 1 - protein, 18 aa, synthetic construct
  REGION 1..18: note = peptide
LKKNGSCKRGPRTHYGQK

SEQ ID NO: 2 - DNA, 20 bp, synthetic construct
  misc_feature 1..20: note = Col1a1-F
  source 1..20: mol_type = other DNA
caccctcaagagcctgagtc

SEQ ID NO: 3 - DNA, 20 bp, synthetic construct
  misc_feature 1..20: note = Col1a1-R
  source 1..20: mol_type = other DNA
agacggctgagtagggaaca

SEQ ID NO: 4 - DNA, 20 bp, synthetic construct
  misc_feature 1..20: note = Fibronectin-F
  source 1..20: mol_type = other DNA
ccaggaaccgagtacaccat

SEQ ID NO: 5 - DNA, 20 bp, synthetic construct
  misc_feature 1..20: note = Fibronectin-R
  source 1..20: mol_type = other DNA
atacccaggttgggtgatga

SEQ ID NO: 6 - DNA, 20 bp, synthetic construct
  misc_feature 1..20: note = Elastin-F
  source 1..20: mol_type = other DNA
gcaagacctggctttggact

SEQ ID NO: 7 - DNA, 21 bp, synthetic construct
  misc_feature 1..21: note = Elastin-R
  source 1..21: mol_type = other DNA
gggagtttctggttagggctg

SEQ ID NO: 8 - DNA, 20 bp, synthetic construct
  misc_feature 1..20: note = GAPDH-F
  source 1..20: mol_type = other DNA
ggagccaaaagggtcatcat

SEQ ID NO: 9 - DNA, 20 bp, synthetic construct
  misc_feature 1..20: note = GAPDH-R
  source 1..20: mol_type = other DNA
gtgatggcatggactgtggt